European Patent Specification EP 3 564 378 B1, published November 1, 2023. Title: Immunogenic Composition. Applicant: GlaxoSmithKline Biologicals s.a. The sequence listing filed with the application follows.

SEQUENCE LISTING (35 sequences)

SEQ ID NO: 1 - protein, 2710 aa, Clostridium Difficile
MSLISKEELIKLAYSIRPRENEYKTILTNLDEYNKLTTNNNENKYLQLKKLNESIDVFMNKYKTSSRNRALSNLKKDILKEVILIKNSNTSPVEKNLHFVWIGGEVSDIALEYIKQWADINAEYNIKLWYDSEAFLVNTLKKAIVESSTTEALQLLEEEIQNPQFDNMKFYKKRMEFIYDRQKRFINYYKSQINKPTVPTIDDIIKSHLVSEYNRDETVLESYRTNSLRKINSNHGIDIRANSLFTEQELLNIYSQELLNRGNLAAASDIVRLLALKNFGGVYLDVDMLPGIHSDLFKTISRPSSIGLDRWEMIKLEAIMKYKKYINNYTSENFDKLDQQLKDNFKLIIESKSEKSEIFSKLENLNVSDLEIKIAFALGSVINQALISKQGSYLTNLVIEQVKNRYQFLNQHLNPAIESDNNFTDTTKIFHDSLFNSATAENSMFLTKIAPYLQVGFMPEARSTISLSGPGAYASAYYDFINLQENTIEKTLKASDLIEFKFPENNLSQLTEQEINSLWSFDQASAKYQFEKYVRDYTGGSLSEDNGVDFNKNTALDKNYLLNNKIPSNNVEEAGSKNYVHYIIQLQGDDISYEATCNLFSKNPKNSIIIQRNMNESAKSYFLSDDGESILELNKYRIPERLKNKEKVKVTFIGHGKDEFNTSEFARLSVDSLSNEISSFLDTIKLDISPKNVEVNLLGCNMFSYDFNVEETYPGKLLLSIMDKITSTLPDVNKNSITIGANQYEVRINSEGRKELLAHSGKWINKEEAIMSDLSSKEYIFFDSIDNKLKAKSKNIPGLASISEDIKTLLLDASVSPDTKFILNNLKLNIESSIGDYIYYEKLEPVKNIIHNSIDDLIDEFNLLENVSDELYELKKLNNLDEKYLISFEDISKNNSTYSVRFINKSNGESVYVETEKEIFSKYSEHITKEISTIKNSIITDVNGNLLDNIQLDHTSQVNTLNAAFFIQSLIDYSSNKDVLNDLSTSVKVQLYAQLFSTGLNTIYDSIQLVNLISNAVNDTINVLPTITEGIPIVSTILDGINLGAAIKELLDEHDPLLKKELEAKVGVLAINMSLSIAATVASIVGIGAEVTIFLLPIAGISAGIPSLVNNELILHDKATSVVNYFNHLSESKKYGPLKTEDDKILVPIDDLVISEIDFNNNSIKLGTCNILAMEGGSGHTVTGNIDHFFSSPSISSHIPSLSIYSAIGIETENLDFSKKIMMLPNAPSRVFWWETGAVPGLRSLENDGTRLLDSIRDLYPGKFYWRFYAFFDYAITTLKPVYEDTNIKIKLDKDTRNFIMPTITTNEIRNKLSYSFDGAGGTYSLLLSSYPISTNINLSKDDLWIFNIDNEVREISIENGTIKKGKLIKDVLSKIDINKNKLIIGNQTIDFSGDIDNKDRYIFLTCELDDKISLIIEINLVAKSYSLLLSGDKNYLISNLSNTIEKINTLGLDSKNIAYNYTDESNNKYFGAISKTSQKSIIHYKKDSKNILEFYNDSTLEFNSKDFIAEDINVFMKDDINTITGKYYVDNNTDKSIDFSISLVSKNQVKVNGLYLNESVYSSYLDFVKNSDGHHNTSNFMNLFLDNISFWKLFGFENINFVIDKYFTLVGKTNLGYVEFICDNNKNIDIYFGEWKTSSSKSTIFSGNGRNVVVEPIYNPDTGEDISTSLDFSYEPLYGIDRYINKVLIAPDLYTSLININTNYYSNEYYPEIIVLNPNTFHKKVNINLDSSSFEYKWSTEGSDFILVRYLEESNKKILQKIRIKGILSNTQSFNKMSIDFKDIKKLSLGYIMSNFKSFNSENELDRDHLGFKIIDNKTYYYDEDSKLVKGLININNSLFYFDPIEFNLVTGWQTINGKKYYFDINTGAALTSYKIINGKHFYFNNDGVMQLGVFKGPDGFEYFAPANTQNNNIEGQAIVYQSKFLTLNGKKYYFDNNSKAVTGWRIINNEKYYFNPNNAIAAVGLQVIDNNKYYFNPDTAIISKGWQTVNGSRYYFDTDTAIAFNGYKTIDGKHFYFDSDCVVKIGVFSTSNGFEYFAPANTYNNNIEGQAIVYQSKFLTLNGKKYYFDNNSKAVTGLQTIDSKKYYFNTNTAEAATGWQTIDGKKYYFNTNTAEAATGWQTIDGKKYYFNTNTAIASTGYTIINGKHFYFNTDGIMQIGVFKGPNGFEYFAPANTDANNIEGQAILYQNEFLTLNGKKYYFGSDSKAVTGWRIINNKKYYFNPNNAIAAIHLCTINNDKYYFSYDGILQNGYITIERNNFYFDANNESKMVTGVFKGPNGFEYFAPANTHNNNIEGQAIVYQNKFLTLNGKKYYFDNDSKAVTGWQTIDGKKYYFNLNTAEAATGWQTIDGKKYYFNLNTAEAATGWQTIDGKKYYFNTNTFIASTGYTSINGKHFYFNTDGIMQIGVFKGPNGFEYFAPANTDANNIEGQAILYQNKFLTLNGKKYYFGSDSKAVTGLRTIDGKKYYFNTNTAVAVTGWQTINGKKYYFNTNTSIASTGYTIISGKHFYFNTDGIMQIGVFKGPDGFEYFAPANTDANNIEGQAIRYQNRFLYLHDNIYYFGNNSKAATGWVTIDGNRYYFEPNTAMGANGYKTIDNKNFYFRNGLPQIGVFKGSNGFEYFAPANTDANNIEGQAIRYQNRFLHLLGKIYYFGNNSKAVTGWQTINGKVYYFMPDTAMAAAGGLFEIDGVIYFFGVDGVKAPGIYG

SEQ ID NO: 2 - protein, 2366 aa, Clostridium Difficile
MSLVNRKQLEKMANVRFRTQEDEYVAILDALEEYHNMSENTVVEKYLKLKDINSLTDIYIDTYKKSGRNKALKKFKEYLVTEVLELKNNNLTPVEKNLHFVWIGGQINDTAINYINQWKDVNSDYNVNVFYDSNAFLINTLKKTVVESAINDTLESFRENLNDPRFDYNKFFRKRMEIIYDKQKNFINYYKAQREENPELIIDDIVKTYLSNEYSKEIDELNTYIEESLNKITQNSGNDVRNFEEFKNGESFNLYEQELVERWNLAAASDILRISALKEIGGMYLDVDMLPGIQPDLFESIEKPSSVTVDFWEMTKLEAIMKYKEYIPEYTSEHFDMLDEEVQSSFESVLASKSDKSEIFSSLGDMEASPLEVKIAFNSKGIINQGLISVKDSYCSNLIVKQIENRYKILNNSLNPAISEDNDFNTTTNTFIDSIMAEANADNGRFMMELGKYLRVGFFPDVKTTINLSGPEAYAAAYQDLLMFKEGSMNIHLIEADLRNFEISKTNISQSTEQEMASLWSFDDARAKAQFEEYKRNYFEGSLGEDDNLDFSQNIVVDKEYLLEKISSLARSSERGYIHYIVQLQGDKISYEAACNLFAKTPYDSVLFQKNIEDSEIAYYYNPGDGEIQEIDKYKIPSIISDRPKIKLTFIGHGKDEFNTDIFAGFDVDSLSTEIEAAIDLAKEDISPKSIEINLLGCNMFSYSINVEETYPGKLLLKVKDKISELMPSISQDSIIVSANQYEVRINSEGRRELLDHSGEWINKEESIIKDISSKEYISFNPKENKITVKSKNLPELSTLLQEIRNNSNSSDIELEEKVMLTECEINVISNIDTQIVEERIEEAKNLTSDSINYIKDEFKLIESISDALCDLKQQNELEDSHFISFEDISETDEGFSIRFINKETGESIFVETEKTIFSEYANHITEEISKIKGTIFDTVNGKLVKKVNLDTTHEVNTLNAAFFIQSLIEYNSSKESLSNLSVAMKVQVYAQLFSTGLNTITDAAKVVELVSTALDETIDLLPTLSEGLPIIATIIDGVSLGAAIKELSETSDPLLRQEIEAKIGIMAVNLTTATTAIITSSLGIASGFSILLVPLAGISAGIPSLVNNELVLRDKATKVVDYFKHVSLVETEGVFTLLDDKIMMPQDDLVISEIDFNNNSIVLGKCEIWRMEGGSGHTVTDDIDHFFSAPSITYREPHLSIYDVLEVQKEELDLSKDLMVLPNAPNRVFAWETGWTPGLRSLENDGTKLLDRIRDNYEGEFYWRYFAFIADALITTLKPRYEDTNIRINLDSNTRSFIVPIITTEYIREKLSYSFYGSGGTYALSLSQYNMGINIELSESDVWIIDVDNVVRDVTIESDKIKKGDLIEGILSTLSIEENKIILNSHEINFSGEVNGSNGFVSLTFSILEGINAIIEVDLLSKSYKLLISGELKILMLNSNHIQQKIDYIGFNSELQKNIPYSFVDSEGKENGFINGSTKEGLFVSELPDVVLISKVYMDDSKPSFGYYSNNLKDVKVITKDNVNILTGYYLKDDIKISLSLTLQDEKTIKLNSVHLDESGVAEILKFMNRKGNTNTSDSLMSFLESMNIKSIFVNFLQSNIKFILDANFIISGTTSIGQFEFICDENDNIQPYFIKFNTLETNYTLYVGNRQNMIVEPNYDLDDSGDISSTVINFSQKYLYGIDSCVNKVVISPNIYTDEINITPVYETNNTYPEVIVLDANYINEKINVNINDLSIRYVWSNDGNDFILMSTSEENKVSQVKIRFVNVFKDKTLANKLSFNFSDKQDVPVSEIILSFTPSYYEDGLIGYDLGLVSLYNEKFYINNFGMMVSGLIYINDSLYYFKPPVNNLITGFVTVGDDKYYFNPINGGAASIGETIIDDKNYYFNQSGVLQTGVFSTEDGFKYFAPANTLDENLEGEAIDFTGKLIIDENIYYFDDNYRGAVEWKELDGEMHYFSPETGKAFKGLNQIGDYKYYFNSDGVMQKGFVSINDNKHYFDDSGVMKVGYTEIDGKHFYFAENGEMQIGVFNTEDGFKYFAHHNEDLGNEEGEEISYSGILNFNNKIYYFDDSFTAVVGWKDLEDGSKYYFDEDTAEAYIGLSLINDGQYYFNDDGIMQVGFVTINDKVFYFSDSGIIESGVQNIDDNYFYIDDNGIVQIGVFDTSDGYKYFAPANTVNDNIYGQAVEYSGLVRVGEDVYYFGETYTIETGWIYDMENESDKYYFNPETKKACKGINLIDDIKYYFDEKGIMRTGLISFENNNYYFNENGEMQFGYINIEDKMFYFGEDGVMQIGVFNTPDGFKYFAHQNTLDENFEGESINYTGWLDLDEKRYYFTDEYIAATGSVIIDGEEYYFDPDTAQLVISE

SEQ ID NO: 3 - protein, 966 aa, Clostridium Difficile
MGWQTIDGKKYYFNTNTAIASTGYTIINGKHFYFNTDGIMQIGVFKGPNGFEYFAPANTDANNIEGQAILYQNEFLTLNGKKYYFGSDSKAVTGWRIINNKKYYFNPNNAIAAIHLCTINNDKYYFSYDGILQNGYITIERNNFYFDANNESKMVTGVFKGPNGFEYFAPANTHNNNIEGQAIVYQNKFLTLNGKKYYFDNDSKAVTGWQTIDGKKYYFNLNTAEAATGWQTIDGKKYYFNLNTAEAATGWQTIDGKKYYFNTNTFIASTGYTSINGKHFYFNTDGIMQIGVFKGPNGFEYFAPANTDANNIEGQAILYQNKFLTLNGKKYYFGSDSKAVTGLRTIDGKKYYFNTNTAVAVTGWQTINGKKYYFNTNTSIASTGYTIISGKHFYFNTDGIMQIGVFKGPDGFEYFAPANTDANNIEGQAIRYQNRFLYLHDNIYYFGNNSKAATGWVTIDGNRYYFEPNTAMGANGYKTIDNKNFYFRNGLPQIGVFKGSNGFEYFAPANTDANNIEGQAIRYQNRFLHLLGKIYYFGNNSKAVTGWQTINGKVYYFMPDTAMAAAGGLFEIDGVIYFFGVDGVKAPGFVSINDNKHYFDDSGVMKVGYTEIDGKHFYFAENGEMQIGVFNTEDGFKYFAHHNEDLGNEEGEEISYSGILNFNNKIYYFDDSFTAVVGWKDLEDGSKYYFDEDTAEAYIGLSLINDGQYYFNDDGIMQVGFVTINDKVFYFSDSGIIESGVQNIDDNYFYIDDNGIVQIGVFDTSDGYKYFAPANTVNDNIYGQAVEYSGLVRVGEDVYYFGETYTIETGWIYDMENESDKYYFNPETKKACKGINLIDDIKYYFDEKGIMRTGLISFENNNYYFNENGEMQFGYINIEDKMFYFGEDGVMQIGVFNTPDGFKYFAHQNTLDENFEGESINYTGWLDLDEKRYYFTDEYIAATGSVIIDGEEYYFDPDTAQLVISE

SEQ ID NO: 4 - protein, 966 aa, Clostridium Difficile
MGWQTIDGKKYYFNTNTAIASTGYTIINGKHFYFNTDGIMQIGVFKGPNGFEYFAPANTDANNIEGQAILYQNEFLTLNGKKYYFGSDSKAVTGWRIINNKKYYFNPNNAIAAIHLCTINNDKYYFSYDGILQNGYITIERNNFYFDANNESKMVTGVFKGPNGFEYFAPANTHNNNIEGQAIVYQNKFLTLNGKKYYFDNDSKAVTGWQTIDGKKYYFNLNTAEAATGWQTIDGKKYYFNLNTAEAATGWQTIDGKKYYFNTNTFIASTGYTSINGKHFYFNTDGIMQIGVFKGPNGFEYFAPANTDANNIEGQAILYQNKFLTLNGKKYYFGSDSKAVTGLRTIDGKKYYFNTNTAVAVTGWQTINGKKYYFNTNTSIASTGYTIISGKHFYFNTDGIMQIGVFKGPDGFEYFAPANTDANNIEGQAIRYQNRFLYLHDNIYYFGNNSKAATGWVTIDGNRYYFEPNTAMGANGYKTIDNKNFYFRNGLPQIGVFKGSNGFEYFAPANTDANNIEGQAIRYQNRFLHLLGKIYYFGNNSKAVTGWQTINGKVYYFMPDTAMAAAGGLNQIGDYKYYFNSDGVMQKGFVSINDNKHYFDDSGVMKVGYTEIDGKHFYFAENGEMQIGVFNTEDGFKYFAHHNEDLGNEEGEEISYSGILNFNNKIYYFDDSFTAVVGWKDLEDGSKYYFDEDTAEAYIGLSLINDGQYYFNDDGIMQVGFVTINDKVFYFSDSGIIESGVQNIDDNYFYIDDNGIVQIGVFDTSDGYKYFAPANTVNDNIYGQAVEYSGLVRVGEDVYYFGETYTIETGWIYDMENESDKYYFNPETKKACKGINLIDDIKYYFDEKGIMRTGLISFENNNYYFNENGEMQFGYINIEDKMFYFGEDGVMQIGVFNTPDGFKYFAHQNTLDENFEGESINYTGWLDLDEKRYYFTDEYIAATGSVIIDGEEYYFDPDTAQLVISE

SEQ ID NO: 5 - protein, 833 aa, Clostridium Difficile
MGWQTIDGKKYYFNTNTAIASTGYTIINGKHFYFNTDGIMQIGVFKGPNGFEYFAPANTDANNIEGQAILYQNEFLTLNGKKYYFGSDSKAVTGWRIINNKKYYFNPNNAIAAIHLCTINNDKYYFSYDGILQNGYITIERNNFYFDANNESKMVTGVFKGPNGFEYFAPANTHNNNIEGQAIVYQNKFLTLNGKKYYFDNDSKAVTGWQTIDGKKYYFNLNTAEAATGWQTIDGKKYYFNLNTAEAATGWQTIDGKKYYFNTNTFIASTGYTSINGKHFYFNTDGIMQIGVFKGPNGFEYFAPANTDANNIEGQAILYQNKFLTLNGKKYYFGSDSKAVTGLRTIDGKKYYFNTNTAVAVTGWQTINGKKYYFNTNTSIASTGYTIISGKHFYFNTDGIMQIGVFKGPDGFEYFAPANTDANNIEGQAIRYQNRFLYLHDNIYYFGNNSKAATGWVTIDGNRYYFEPNTAMGANGYKTIDNKNFYFRNGLPQIGVFKGSNGFEYFAHHNEDLGNEEGEEISYSGILNFNNKIYYFDDSFTAVVGWKDLEDGSKYYFDEDTAEAYIGLSLINDGQYYFNDDGIMQVGFVTINDKVFYFSDSGIIESGVQNIDDNYFYIDDNGIVQIGVFDTSDGYKYFAPANTVNDNIYGQAVEYSGLVRVGEDVYYFGETYTIETGWIYDMENESDKYYFNPETKKACKGINLIDDIKYYFDEKGIMRTGLISFENNNYYFNENGEMQFGYINIEDKMFYFGEDGVMQIGVFNTPDGFKYFAHQNTLDENFEGESINYTGWLDLDEKRYYFTDEYIAATGSVIIDGEEYYFDPDTAQLVISE

SEQ ID NO: 6 - protein, 1057 aa, Clostridium Difficile
MGWQTIDGKKYYFNTNTAIASTGYTIINGKHFYFNTDGIMQIGVFKGPNGFEYFAPANTDANNIEGQAILYQNEFLTLNGKKYYFGSDSKAVTGWRIINNKKYYFNPNNAIAAIHLCTINNDKYYFSYDGILQNGYITIERNNFYFDANNESKMVTGVFKGPNGFEYFAPANTHNNNIEGQAIVYQNKFLTLNGKKYYFDNDSKAVTGWQTIDGKKYYFNLNTAEAATGWQTIDGKKYYFNLNTAEAATGWQTIDGKKYYFNTNTFIASTGYTSINGKHFYFNTDGIMQIGVFKGPNGFEYFAPANTDANNIEGQAILYQNKFLTLNGKKYYFGSDSKAVTGLRTIDGKKYYFNTNTAVAVTGWQTINGKKYYFNTNTSIASTGYTIISGKHFYFNTDGIMQIGVFKGPDGFEYFAPANTDANNIEGQAIRYQNRFLYLHDNIYYFGNNSKAATGWVTIDGNRYYFEPNTAMGANGYKTIDNKNFYFRNGLPQIGVFKGSNGFEYFAPANTDANNIEGQAIRYQNRFLHLLGKIYYFGNNSKAVTGWQTINGKVYYFMPDTAMAAAGGETIIDDKNYYFNQSGVLQTGVFSTEDGFKYFAPANTLDENLEGEAIDFTGKLIIDENIYYFDDNYRGAVEWKELDGEMHYFSPETGKAFKGLNQIGDYKYYFNSDGVMQKGFVSINDNKHYFDDSGVMKVGYTEIDGKHFYFAENGEMQIGVFNTEDGFKYFAHHNEDLGNEEGEEISYSGILNFNNKIYYFDDSFTAVVGWKDLEDGSKYYFDEDTAEAYIGLSLINDGQYYFNDDGIMQVGFVTINDKVFYFSDSGIIESGVQNIDDNYFYIDDNGIVQIGVFDTSDGYKYFAPANTVNDNIYGQAVEYSGLVRVGEDVYYFGETYTIETGWIYDMENESDKYYFNPETKKACKGINLIDDIKYYFDEKGIMRTGLISFENNNYYFNENGEMQFGYINIEDKMFYFGEDGVMQIGVFNTPDGFKYFAHQNTLDENFEGESINYTGWLDLDEKRYYFTDEYIAATGSVIIDGEEYYFDPDTAQLVISE

SEQ ID NO: 7 - protein, 971 aa, Clostridium Difficile
MGWQTIDGKKYYFNTNTAIASTGYTIINGKHFYFNTDGIMQIGVFKGPNGFEYFAPANTDANNIEGQAILYQNEFLTLNGKKYYFGSDSKAVTGWRIINNKKYYFNPNNAIAAIHLCTINNDKYYFSYDGILQNGYITIERNNFYFDANNESKMVTGVFKGPNGFEYFAPANTHNNNIEGQAIVYQNKFLTLNGKKYYFDNDSKAVTGWQTIDGKKYYFNLNTAEAATGWQTIDGKKYYFNLNTAEAATGWQTIDGKKYYFNTNTFIASTGYTSINGKHFYFNTDGIMQIGVFKGPNGFEYFAPANTDANNIEGQAILYQNKFLTLNGKKYYFGSDSKAVTGLRTIDGKKYYFNTNTAVAVTGWQTINGKKYYFNTNTSIASTGYTIISGKHFYFNTDGIMQIGVFKGPDGFEYFAPANTDANNIEGQAIRYQNRFLYLHDNIYYFGNNSKAATGWVTIDGNRYYFEPNTAMGANGYKTIDNKNFYFRNGLPQIGVFKGSNGFEYFAPANTDANNIEGQAIRYQNRFLHLLGKIYYFGNNSKAVTGWQTINGKVYYFMPDTAMAAAGGLFEIDGVIYFFGVDGVKAPGIYGGGFVSINDNKHYFDDSGVMKVGYTEIDGKHFYFAENGEMQIGVFNTEDGFKYFAHHNEDLGNEEGEEISYSGILNFNNKIYYFDDSFTAVVGWKDLEDGSKYYFDEDTAEAYIGLSLINDGQYYFNDDGIMQVGFVTINDKVFYFSDSGIIESGVQNIDDNYFYIDDNGIVQIGVFDTSDGYKYFAPANTVNDNIYGQAVEYSGLVRVGEDVYYFGETYTIETGWIYDMENESDKYYFNPETKKACKGINLIDDIKYYFDEKGIMRTGLISFENNNYYFNENGEMQFGYINIEDKMFYFGEDGVMQIGVFNTPDGFKYFAHQNTLDENFEGESINYTGWLDLDEKRYYFTDEYIAATGSVIIDGEEYYFDPDTAQLVISE

SEQ ID NO: 8 - protein, 321 aa, Clostridium Difficile
MASTGYTSINGKHFYFNTDGIMQIGVFKGPNGFEYFAPANTDANNIEGQAILYQNKFLTLNGKKYYFGSDSKAVTGLRTIDGKKYYFNTNTAVAVTGWQTINGKKYYFNTNTSIASTGYTIISGKHFYFNTDGIMQIGVFKGPDGFEYFAPANTDANNIEGQAIRYQNRFLYLHDNIYYFGNNSKAATGWVTIDGNRYYFEPNTAMGANGYKTIDNKNFYFRNGLPQIGVFKGSNGFEYFAPANTDANNIEGQAIRYQNRFLHLLGKIYYFGNNSKAVTGWQTINGKVYYFMPDTAMAAAGGLFEIDGVIYFFGVDGVKAP

SEQ ID NO: 9 - protein, 612 aa, Clostridium Difficile
MILMSTSEENKVSQVKIRFVNVFKDKTLANKLSFNFSDKQDVPVSEIILSFTPSYYEDGLIGYDLGLVSLYNEKFYINNFGMMVSGLIYINDSLYYFKPPVNNLITGFVTVGDDKYYFNPINGGAASIGETIIDDKNYYFNQSGVLQTGVFSTEDGFKYFAPANTLDENLEGEAIDFTGKLIIDENIYYFDDNYRGAVEWKELDGEMHYFSPETGKAFKGLNQIGDYKYYFNSDGVMQKGFVSINDNKHYFDDSGVMKVGYTEIDGKHFYFAENGEMQIGVFNTEDGFKYFAHHNEDLGNEEGEEISYSGILNFNNKIYYFDDSFTAVVGWKDLEDGSKYYFDEDTAEAYIGLSLINDGQYYFNDDGIMQVGFVTINDKVFYFSDSGIIESGVQNIDDNYFYIDDNGIVQIGVFDTSDGYKYFAPANTVNDNIYGQAVEYSGLVRVGEDVYYFGETYTIETGWIYDMENESDKYYFNPETKKACKGINLIDDIKYYFDEKGIMRTGLISFENNNYYFNENGEMQFGYINIEDKMFYFGEDGVMQIGVFNTPDGFKYFAHQNTLDENFEGESINYTGWLDLDEKRYYFTDEYIAATGSVIIDGEEYYFDPDTA

SEQ ID NO: 10 - protein, 587 aa, Clostridium Difficile
MGWQTIDGKKYYFNTNTAIASTGYTIINGKHFYFNTDGIMQIGVFKGPNGFEYFAPANTDANNIEGQAILYQNEFLTLNGKKYYFGSDSKAVTGWRIINNKKYYFNPNNAIAAIHLCTINNDKYYFSYDGILQNGYITIERNNFYFDANNESKMVTGVFKGPNGFEYFAPANTHNNNIEGQAIVYQNKFLTLNGKKYYFDNDSKAVTGWQTIDGKKYYFNLNTAEAATGWQTIDGKKYYFNLNTAEAATGWQTIDGKKYYFNTNTFIASTGYTSINGKHFYFNTDGIMQIGVFKGPNGFEYFAPANTDANNIEGQAILYQNKFLTLNGKKYYFGSDSKAVTGLRTIDGKKYYFNTNTAVAVTGWQTINGKKYYFNTNTSIASTGYTIISGKHFYFNTDGIMQIGVFKGPDGFEYFAPANTDANNIEGQAIRYQNRFLYLHDNIYYFGNNSKAATGWVTIDGNRYYFEPNTAMGANGYKTIDNKNFYFRNGLPQIGVFKGSNGFEYFAPANTDANNIEGQAIRYQNRFLHLLGKIYYFGNNSKAVTGWQTINGKVYYFMPDTAMAAAGGLFEIDGVIYFFGVDGVKAP

SEQ ID NO: 11 - protein, 567 aa, Clostridium Difficile
MGWQTIDGKKYYFNTNTAIASTGYTIINGKHFYFNTDGIMQIGVFKGPNGFEYFAPANTDANNIEGQAILYQNEFLTLNGKKYYFGSDSKAVTGWRIINNKKYYFNPNNAIAAIHLCTINNDKYYFSYDGILQNGYITIERNNFYFDANNESKMVTGVFKGPNGFEYFAPANTHNNNIEGQAIVYQNKFLTLNGKKYYFDNDSKAVTGWQTIDGKKYYFNLNTAEAATGWQTIDGKKYYFNLNTAEAATGWQTIDGKKYYFNTNTFIASTGYTSINGKHFYFNTDGIMQIGVFKGPNGFEYFAPANTDANNIEGQAILYQNKFLTLNGKKYYFGSDSKAVTGLRTIDGKKYYFNTNTAVAVTGWQTINGKKYYFNTNTSIASTGYTIISGKHFYFNTDGIMQIGVFKGPDGFEYFAPANTDANNIEGQAIRYQNRFLYLHDNIYYFGNNSKAATGWVTIDGNRYYFEPNTAMGANGYKTIDNKNFYFRNGLPQIGVFKGSNGFEYFAPANTDANNIEGQAIRYQNRFLHLLGKIYYFGNNSKAVTGWQTINGKVYYFMPDTAMAAAG

SEQ ID NO: 12 - protein, 505 aa, Clostridium Difficile
MGWQTIDGKKYYFNTNTAIASTGYTIINGKHFYFNTDGIMQIGVFKGPNGFEYFAPANTDANNIEGQAILYQNEFLTLNGKKYYFGSDSKAVTGWRIINNKKYYFNPNNAIAAIHLCTINNDKYYFSYDGILQNGYITIERNNFYFDANNESKMVTGVFKGPNGFEYFAPANTHNNNIEGQAIVYQNKFLTLNGKKYYFDNDSKAVTGWQTIDGKKYYFNLNTAEAATGWQTIDGKKYYFNLNTAEAATGWQTIDGKKYYFNTNTFIASTGYTSINGKHFYFNTDGIMQIGVFKGPNGFEYFAPANTDANNIEGQAILYQNKFLTLNGKKYYFGSDSKAVTGLRTIDGKKYYFNTNTAVAVTGWQTINGKKYYFNTNTSIASTGYTIISGKHFYFNTDGIMQIGVFKGPDGFEYFAPANTDANNIEGQAIRYQNRFLYLHDNIYYFGNNSKAATGWVTIDGNRYYFEPNTAMGANGYKTIDNKNFYFRNGLPQIGVFKGSNGFEY

SEQ ID NO: 13 - protein, 567 aa, Clostridium Difficile; identical to SEQ ID NO: 11

SEQ ID NO: 14 - protein, 591 aa, Clostridium Difficile
MGWQTIDGKKYYFNTNTAIASTGYTIINGKHFYFNTDGIMQIGVFKGPNGFEYFAPANTDANNIEGQAILYQNEFLTLNGKKYYFGSDSKAVTGWRIINNKKYYFNPNNAIAAIHLCTINNDKYYFSYDGILQNGYITIERNNFYFDANNESKMVTGVFKGPNGFEYFAPANTHNNNIEGQAIVYQNKFLTLNGKKYYFDNDSKAVTGWQTIDGKKYYFNLNTAEAATGWQTIDGKKYYFNLNTAEAATGWQTIDGKKYYFNTNTFIASTGYTSINGKHFYFNTDGIMQIGVFKGPNGFEYFAPANTDANNIEGQAILYQNKFLTLNGKKYYFGSDSKAVTGLRTIDGKKYYFNTNTAVAVTGWQTINGKKYYFNTNTSIASTGYTIISGKHFYFNTDGIMQIGVFKGPDGFEYFAPANTDANNIEGQAIRYQNRFLYLHDNIYYFGNNSKAATGWVTIDGNRYYFEPNTAMGANGYKTIDNKNFYFRNGLPQIGVFKGSNGFEYFAPANTDANNIEGQAIRYQNRFLHLLGKIYYFGNNSKAVTGWQTINGKVYYFMPDTAMAAAGGLFEIDGVIYFFGVDGVKAPGIYG

SEQ ID NO: 15 - protein, 379 aa, Clostridium Difficile
GFVSINDNKHYFDDSGVMKVGYTEIDGKHFYFAENGEMQIGVFNTEDGFKYFAHHNEDLGNEEGEEISYSGILNFNNKIYYFDDSFTAVVGWKDLEDGSKYYFDEDTAEAYIGLSLINDGQYYFNDDGIMQVGFVTINDKVFYFSDSGIIESGVQNIDDNYFYIDDNGIVQIGVFDTSDGYKYFAPANTVNDNIYGQAVEYSGLVRVGEDVYYFGETYTIETGWIYDMENESDKYYFNPETKKACKGINLIDDIKYYFDEKGIMRTGLISFENNNYYFNENGEMQFGYINIEDKMFYFGEDGVMQIGVFNTPDGFKYFAHQNTLDENFEGESINYTGWLDLDEKRYYFTDEYIAATGSVIIDGEEYYFDPDTAQLVISE

SEQ ID NO: 16 - protein, 399 aa, Clostridium Difficile
GLNQIGDYKYYFNSDGVMQKGFVSINDNKHYFDDSGVMKVGYTEIDGKHFYFAENGEMQIGVFNTEDGFKYFAHHNEDLGNEEGEEISYSGILNFNNKIYYFDDSFTAVVGWKDLEDGSKYYFDEDTAEAYIGLSLINDGQYYFNDDGIMQVGFVTINDKVFYFSDSGIIESGVQNIDDNYFYIDDNGIVQIGVFDTSDGYKYFAPANTVNDNIYGQAVEYSGLVRVGEDVYYFGETYTIETGWIYDMENESDKYYFNPETKKACKGINLIDDIKYYFDEKGIMRTGLISFENNNYYFNENGEMQFGYINIEDKMFYFGEDGVMQIGVFNTPDGFKYFAHQNTLDENFEGESINYTGWLDLDEKRYYFTDEYIAATGSVIIDGEEYYFDPDTAQLVISE

SEQ ID NO: 17 - protein, 328 aa, Clostridium Difficile
FAHHNEDLGNEEGEEISYSGILNFNNKIYYFDDSFTAVVGWKDLEDGSKYYFDEDTAEAYIGLSLINDGQYYFNDDGIMQVGFVTINDKVFYFSDSGIIESGVQNIDDNYFYIDDNGIVQIGVFDTSDGYKYFAPANTVNDNIYGQAVEYSGLVRVGEDVYYFGETYTIETGWIYDMENESDKYYFNPETKKACKGINLIDDIKYYFDEKGIMRTGLISFENNNYYFNENGEMQFGYINIEDKMFYFGEDGVMQIGVFNTPDGFKYFAHQNTLDENFEGESINYTGWLDLDEKRYYFTDEYIAATGSVIIDGEEYYFDPDTAQLVISE

SEQ ID NO: 18 - protein, 490 aa, Clostridium Difficile
GETIIDDKNYYFNQSGVLQTGVFSTEDGFKYFAPANTLDENLEGEAIDFTGKLIIDENIYYFDDNYRGAVEWKELDGEMHYFSPETGKAFKGLNQIGDYKYYFNSDGVMQKGFVSINDNKHYFDDSGVMKVGYTEIDGKHFYFAENGEMQIGVFNTEDGFKYFAHHNEDLGNEEGEEISYSGILNFNNKIYYFDDSFTAVVGWKDLEDGSKYYFDEDTAEAYIGLSLINDGQYYFNDDGIMQVGFVTINDKVFYFSDSGIIESGVQNIDDNYFYIDDNGIVQIGVFDTSDGYKYFAPANTVNDNIYGQAVEYSGLVRVGEDVYYFGETYTIETGWIYDMENESDKYYFNPETKKACKGINLIDDIKYYFDEKGIMRTGLISFENNNYYFNENGEMQFGYINIEDKMFYFGEDGVMQIGVFNTPDGFKYFAHQNTLDENFEGESINYTGWLDLDEKRYYFTDEYIAATGSVIIDGEEYYFDPDTAQLVISE

SEQ ID NO: 19 - protein, 379 aa, Clostridium Difficile; identical to SEQ ID NO: 15

SEQ ID NO: 20 - DNA, 3339 bp, Clostridium Difficile
atggcaaccggttggcagaccatcgatggcaaaaaatattattttaataccaacaccgcaattgcaagcaccggctataccattatcaacggcaaacacttttattttaacaccgacggcattatgcagattggtgtgtttaaaggtccgaacggctttgaatactttgcaccggcaaataccgatgccaataatattgaaggccaggccattctgtatcagaatgaatttctgaccctgaacggcaaaaaatactactttggcagcgatagcaaagcagttaccggttggcgcatcatcaacaataagaaatattacttcaacccgaataatgcaattgcagcaattcatctgtgcaccattaacaacgacaaatattatttcagctatgacggtattctgcagaatggctacattaccatcgaacgcaacaacttttatttcgatgccaacaacgaaagcaaaatggtgaccggtgttttcaaaggccctaatggttttgagtatttcgctccggcaaacacccataataacaacattgaaggtcaggcgatcgtttatcagaacaaattcctgacgctgaatggtaagaaatactatttcgataatgacagcaaagccgtgaccggctggcagacaattgacgggaagaaatattactttaatctgaataccgcagaagcagcaaccggttggcaaacgatcgacggtaaaaagtactacttcaacctgaacacagccgaagcagccacaggatggcagactattgatggaaaaaaatactatttcaacaccaacacctttattgcatctaccggttataccagcattaacggtaaacatttctacttcaacaccgatggtatcatgcagatcggcgttttcaaaggtccaaatggtttcgaatactttgcccctgccaatacagatgcaaataacatcgagggtcaggcaatcctgtaccaaaacaaatttctgaccctgaatgggaaaaaatattactttggtagcgattctaaagccgttaccggtctgcgtaccattgatggtaaaaaatactactttaatacgaatacagccgttgcggttacaggctggcagaccattaacgggaaaaaatactattttaacacaaataccagcattgcctcaacgggttataccattatttcgggtaaacacttctactttaataccgatggtattatgcaaatcggagtctttaaaggacctgatgggttcgaatattttgcgcctgcgaacactgatgcgaacaatatcgaaggacaggcaatccgctatcagaatcgctttctgtatctgcacgacaacatctattattttggcaacaattcaaaagcagccaccggctgggttacaattgatggcaaccgctactatttcgaaccgaataccgcaatgggtgcaaatggctacaaaaccatcgataataaaaatttctattttcgcaacggtctgccgcagatcggggtatttaaaggtagcaacggcttcgaatacttcgctccagcgaatacggacgcgaacaatattgagggtcaagcgattcgttatcaaaaccgttttctgcatctgctgggcaaaatctactactttggcaataacagtaaagcagttactggatggcagacaatcaatggtaaagtgtactattttatgccggataccgccatggcagcagccggtggtctgtttgaaattgatggcgtgatctatttttttggtgtggatggtgttaaagcaccgggaatatacggtggtaccggctttgtgaccgtgggtgatgataaatactatttcaatccgattaacggtggtgcagcgagcattggcgaaaccatcatcgatgacaaaaactattatttcaaccagagcggtgtgctgcagaccggtgtgtttagcaccgaagatggctttaaatattttgcgccagcgaacaccctggatgaaaacctggaaggcgaagcgattgattttaccggcaaactgatcatcgatgaaaacatctattacttcgatgataactatcgtggtgcggtggaatggaaagaactggatggcgaaatgcattatttttctccggaaaccggtaaagcgtttaaaggcctgaaccagatcggcgattacaaatactacttcaacagcgatggcgtgatgcagaaaggctttgtgagcatcaacgataacaaacactatttcgatgatagcggtgtgatgaaagtgggctataccgaaattgatggcaaacatttctacttcgcggaaaacggcgaaatgcagattggcgtgttcaataccgaagatggtttcaaatacttcgcgcaccataacgaagatctgggtaacgaagaaggcgaagaaattagctatagcggcatcctgaacttcaacaacaaaatctactactttgatgatagctttaccgcggtggtgggctggaaagatctggaagatggcagcaaatattatttcgatgaagataccgcggaagcgtatattggcctgagcctgattaacgatggccagtactattttaacgatgatggcattatgcaggtgggtttcgtgaccattaatgataaagtgttctatttcagcgatagcggcattattgaaagcggcgtgcagaacattgatgataactacttctacatcgatgataacggcattgtgcagatcggcgtttttgataccagcgatggctacaaatatttcgcaccggccaataccgtgaacgataacatttatggccaggcggtggaatatagcggtctggtgcgtgtgggcgaagatgtgtattatttcggcgaaacctataccatcgaaaccggctggatttatgatatggaaaacgaaagcgataaatattactttaatccggaaacgaaaaaagcgtgcaaaggcattaacctgatcgatgatatcaaatactattttgatgaaaaaggcattatgcgtaccggtctgattagcttcgaaaacaacaactattacttcaacgaaaacggtgaaatgcagttcggctacatcaacatcgaagataaaatgttctacttcggcgaagatggtgttatgcagattggtgtttttaacaccccggatggcttcaaatactttgcccatcagaataccctggatgaaaatttcgaaggtgaaagcattaactataccggctggctggatctggatgaaaaacgctactacttcaccgatgaatacattgcggcgaccggcagcgtgattattgatggcgaagaatactacttcgatccggataccgcgcagctggtgattagcgaacatcatcatcatcaccat

SEQ ID NO: 21 - protein, 1113 aa, Clostridium Difficile
MATGWQTIDGKKYYFNTNTAIASTGYTIINGKHFYFNTDGIMQIGVFKGPNGFEYFAPANTDANNIEGQAILYQNEFLTLNGKKYYFGSDSKAVTGWRIINNKKYYFNPNNAIAAIHLCTINNDKYYFSYDGILQNGYITIERNNFYFDANNESKMVTGVFKGPNGFEYFAPANTHNNNIEGQAIVYQNKFLTLNGKKYYFDNDSKAVTGWQTIDGKKYYFNLNTAEAATGWQTIDGKKYYFNLNTAEAATGWQTIDGKKYYFNTNTFIASTGYTSINGKHFYFNTDGIMQIGVFKGPNGFEYFAPANTDANNIEGQAILYQNKFLTLNGKKYYFGSDSKAVTGLRTIDGKKYYFNTNTAVAVTGWQTINGKKYYFNTNTSIASTGYTIISGKHFYFNTDGIMQIGVFKGPDGFEYFAPANTDANNIEGQAIRYQNRFLYLHDNIYYFGNNSKAATGWVTIDGNRYYFEPNTAMGANGYKTIDNKNFYFRNGLPQIGVFKGSNGFEYFAPANTDANNIEGQAIRYQNRFLHLLGKIYYFGNNSKAVTGWQTINGKVYYFMPDTAMAAAGGLFEIDGVIYFFGVDGVKAPGIYGGTGFVTVGDDKYYFNPINGGAASIGETIIDDKNYYFNQSGVLQTGVFSTEDGFKYFAPANTLDENLEGEAIDFTGKLIIDENIYYFDDNYRGAVEWKELDGEMHYFSPETGKAFKGLNQIGDYKYYFNSDGVMQKGFVSINDNKHYFDDSGVMKVGYTEIDGKHFYFAENGEMQIGVFNTEDGFKYFAHHNEDLGNEEGEEISYSGILNFNNKIYYFDDSFTAVVGWKDLEDGSKYYFDEDTAEAYIGLSLINDGQYYFNDDGIMQVGFVTINDKVFYFSDSGIIESGVQNIDDNYFYIDDNGIVQIGVFDTSDGYKYFAPANTVNDNIYGQAVEYSGLVRVGEDVYYFGETYTIETGWIYDMENESDKYYFNPETKKACKGINLIDDIKYYFDEKGIMRTGLISFENNNYYFNENGEMQFGYINIEDKMFYFGEDGVMQIGVFNTPDGFKYFAHQNTLDENFEGESINYTGWLDLDEKRYYFTDEYIAATGSVIIDGEEYYFDPDTAQLVISEHHHHHH

SEQ ID NO: 22 - DNA, 3324 bp, Clostridium Difficile
atggcaaccggttggcagaccatcgatggcaaaaaatattattttaataccaacaccgcaattgcaagcaccggctataccattatcaacggcaaacacttttattttaacaccgacggcattatgcagattggtgtgtttaaaggtccgaacggctttgaatactttgcaccggcaaataccgatgccaataatattgaaggccaggccattctgtatcagaatgaatttctgaccctgaacggcaaaaaatactactttggcagcgatagcaaagcagttaccggttggcgcatcatcaacaataagaaatattacttcaacccgaataatgcaattgcagcaattcatctgtgcaccattaacaacgacaaatattatttcagctatgacggtattctgcagaatggctacattaccatcgaacgcaacaacttttatttcgatgccaacaacgaaagcaaaatggtgaccggtgttttcaaaggccctaatggttttgagtatttcgctccggcaaacacccataataacaacattgaaggtcaggcgatcgtttatcagaacaaattcctgacgctgaatggtaagaaatactatttcgataatgacagcaaagccgtgaccggctggcagacaattgacgggaagaaatattactttaatctgaataccgcagaagcagcaaccggttggcaaacgatcgacggtaaaaagtactacttcaacctgaacacagccgaagcagccacaggatggcagactattgatggaaaaaaatactatttcaacaccaacacctttattgcatctaccggttataccagcattaacggtaaacatttctacttcaacaccgatggtatcatgcagatcggcgttttcaaaggtccaaatggtttcgaatactttgcccctgccaatacagatgcaaataacatcgagggtcaggcaatcctgtaccaaaacaaatttctgaccctgaatgggaaaaaatattactttggtagcgattctaaagccgttaccggtctgcgtaccattgatggtaaaaaatactactttaatacgaatacagccgttgcggttacaggctggcagaccattaacgggaaaaaatactattttaacacaaataccagcattgcctcaacgggttataccattatttcgggtaaacacttctactttaataccgatggtattatgcaaatcggagtctttaaaggacctgatgggttcgaatattttgcgcctgcgaacactgatgcgaacaatatcgaaggacaggcaatccgctatcagaatcgctttctgtatctgcacgacaacatctattattttggcaacaattcaaaagcagccaccggctgggttacaattgatggcaaccgctactatttcgaaccgaataccgcaatgggtgcaaatggctacaaaaccatcgataataaaaatttctattttcgcaacggtctgccgcagatcggggtatttaaaggtagcaacggcttcgaatacttcgctccagcgaatacggacgcgaacaatattgagggtcaagcgattcgttatcaaaaccgttttctgcatctgctgggcaaaatctactactttggcaataacagtaaagcagttactggatggcagacaatcaatggtaaagtgtactattttatgccggataccgccatggcagcagccggtggtctgtttgaaattgatggcgtgatctatttttttggtgtggatggtgttaaagcagttaccggctttgtgaccgtgggtgatgataaatactatttcaatccgattaacggtggtgcagcgagcattggcgaaaccatcatcgatgacaaaaactattatttcaaccagagcggtgtgctgcagaccggtgtgtttagcaccgaagatggctttaaatattttgcgccagcgaacaccctggatgaaaacctggaaggcgaagcgattgattttaccggcaaactgatcatcgatgaaaacatctattacttcgatgataactatcgtggtgcggtggaatggaaagaactggatggcgaaatgcattatttttctccggaaaccggtaaagcgtttaaaggcctgaaccagatcggcgattacaaatactacttcaacagcgatggcgtgatgcagaaaggctttgtgagcatcaacgataacaaacactatttcgatgatagcggtgtgatgaaagtgggctataccgaaattgatggcaaacatttctacttcgcggaaaacggcgaaatgcagattggcgtgttcaataccgaagatggtttcaaatacttcgcgcaccataacgaagatctgggtaacgaagaaggcgaagaaattagctatagcggcatcctgaacttcaacaacaaaatctactactttgatgatagctttaccgcggtggtgggctggaaagatctggaagatggcagcaaatattatttcgatgaagataccgcggaagcgtatattggcctgagcctgattaacgatggccagtactattttaacgatgatggcattatgcaggtgggtttcgtgaccattaatgataaagtgttctatttcagcgatagcggcattattgaaagcggcgtgcagaacattgatgataactacttctacatcgatgataacggcattgtgcagatcggcgtttttgataccagcgatggctacaaatatttcgcaccggccaataccgtgaacgataacatttatggccaggcggtggaatatagcggtctggtgcgtgtgggcgaagatgtgtattatttcggcgaaacctataccatcgaaaccggctggatttatgatatggaaaacgaaagcgataaatattactttaatccggaaacgaaaaaagcgtgcaaaggcattaacctgatcgatgatatcaaatactattttgatgaaaaaggcattatgcgtaccggtctgattagcttcgaaaacaacaactattacttcaacgaaaacggtgaaatgcagttcggctacatcaacatcgaagataaaatgttctacttcggcgaagatggtgttatgcagattggtgtttttaacaccccggatggcttcaaatactttgcccatcagaataccctggatgaaaatttcgaaggtgaaagcattaactataccggctggctggatctggatgaaaaacgctactacttcaccgatgaatacattgcggcgaccggcagcgtgattattgatggcgaagaatactacttcgatccggataccgcgcagctggtgattagcgaacatcatcatcatcaccat

SEQ ID NO: 23 - protein, 1108 aa, Clostridium Difficile
MATGWQTIDGKKYYFNTNTAIASTGYTIINGKHFYFNTDGIMQIGVFKGPNGFEYFAPANTDANNIEGQAILYQNEFLTLNGKKYYFGSDSKAVTGWRIINNKKYYFNPNNAIAAIHLCTINNDKYYFSYDGILQNGYITIERNNFYFDANNESKMVTGVFKGPNGFEYFAPANTHNNNIEGQAIVYQNKFLTLNGKKYYFDNDSKAVTGWQTIDGKKYYFNLNTAEAATGWQTIDGKKYYFNLNTAEAATGWQTIDGKKYYFNTNTFIASTGYTSINGKHFYFNTDGIMQIGVFKGPNGFEYFAPANTDANNIEGQAILYQNKFLTLNGKKYYFGSDSKAVTGLRTIDGKKYYFNTNTAVAVTGWQTINGKKYYFNTNTSIASTGYTIISGKHFYFNTDGIMQIGVFKGPDGFEYFAPANTDANNIEGQAIRYQNRFLYLHDNIYYFGNNSKAATGWVTIDGNRYYFEPNTAMGANGYKTIDNKNFYFRNGLPQIGVFKGSNGFEYFAPANTDANNIEGQAIRYQNRFLHLLGKIYYFGNNSKAVTGWQTINGKVYYFMPDTAMAAAGGLFEIDGVIYFFGVDGVKAVTGFVTVGDDKYYFNPINGGAASIGETIIDDKNYYFNQSGVLQTGVFSTEDGFKYFAPANTLDENLEGEAIDFTGKLIIDENIYYFDDNYRGAVEWKELDGEMHYFSPETGKAFKGLNQIGDYKYYFNSDGVMQKGFVSINDNKHYFDDSGVMKVGYTEIDGKHFYFAENGEMQIGVFNTEDGFKYFAHHNEDLGNEEGEEISYSGILNFNNKIYYFDDSFTAVVGWKDLEDGSKYYFDEDTAEAYIGLSLINDGQYYFNDDGIMQVGFVTINDKVFYFSDSGIIESGVQNIDDNYFYIDDNGIVQIGVFDTSDGYKYFAPANTVNDNIYGQAVEYSGLVRVGEDVYYFGETYTIETGWIYDMENESDKYYFNPETKKACKGINLIDDIKYYFDEKGIMRTGLISFENNNYYFNENGEMQFGYINIEDKMFYFGEDGVMQIGVFNTPDGFKYFAHQNTLDENFEGESINYTGWLDLDEKRYYFTDEYIAATGSVIIDGEEYYFDPDTAQLVISEHHHHHH

SEQ ID NO: 24 - DNA, 3387 bp, Clostridium Difficile
atggcaaccggttggcagaccatcgatggcaaaaaatattattttaataccaacaccgcaattgcaagcaccggctataccattatcaacggcaaacacttttattttaacaccgacggcattatgcagattggtgtgtttaaaggtccgaacggctttgaatactttgcaccggcaaataccgatgccaataatattgaaggccaggccattctgtatcagaatgaatttctgaccctgaacggcaaaaaatactactttggcagcgatagcaaagcagttaccggttggcgcatcatcaacaataagaaatattacttcaacccgaataatgcaattgcagcaattcatctgtgcaccattaacaacgacaaatattatttcagctatgacggtattctgcagaatggctacattaccatcgaacgcaacaacttttatttcgatgccaacaacgaaagcaaaatggtgaccggtgttttcaaaggccctaatggttttgagtatttcgctccggcaaacacccataataacaacattgaaggtcaggcgatcgtttatcagaacaaattcctgacgctgaatggtaagaaatactatttcgataatgacagcaaagccgtgaccggctggcagacaattgacgggaagaaatattactttaatctgaataccgcagaagcagcaaccggttggcaaacgatcgacggtaaaaagtactacttcaacctgaacacagccgaagcagccacaggatggcagactattgatggaaaaaaatactatttcaacaccaacacctttattgcatctaccggttataccagcattaacggtaaacatttctacttcaacaccgatggtatcatgcagatcggcgttttcaaaggtccaaatggtttcgaatactttgcccctgccaatacagatgcaaataacatcgagggtcaggcaatcctgtaccaaaacaaatttctgaccctgaatgggaaaaaatattactttggtagcgattctaaagccgttaccggtctgcgtaccattgatggtaaaaaatactactttaatacgaatacagccgttgcggttacaggctggcagaccattaacgggaaaaaatactattttaacacaaataccagcattgcctcaacgggttataccattatttcgggtaaacacttctactttaataccgatggtattatgcaaatcggagtctttaaaggacctgatgggttcgaatattttgcgcctgcgaacactgatgcgaacaatatcgaaggacaggcaatccgctatcagaatcgctttctgtatctgcacgacaacatctattattttggcaacaattcaaaagcagccaccggctgggttacaattgatggcaaccgctactatttcgaaccgaataccgcaatgggtgcaaatggctacaaaaccatcgataataaaaatttctattttcgcaacggtctgccgcagatcggggtatttaaaggtagcaacggcttcgaatacttcgctccagcgaatacggacgcgaacaatattgagggtcaagcgattcgttatcaaaaccgttttctgcatctgctgggcaaaatctactactttggcaataacagtaaagcagttactggatggcagacaatcaatggtaaagtgtactattttatgccggataccgccatggcagcagccggtggtctgtttgaaattgatggcgtgatctatttttttggtgtggatggtgttaaagcagtgagcggtctgatttatattaacgatagcctgtattactttaaaccaccggtgaataacctgattaccggctttgtgaccgtgggtgatgataaatactatttcaatccgattaacggtggtgcagcgagcattggcgaaaccatcatcgatgacaaaaactattatttcaaccagagcggtgtgctgcagaccggtgtgtttagcaccgaagatggctttaaatattttgcgccagcgaacaccctggatgaaaacctggaaggcgaagcgattgattttaccggcaaactgatcatcgatgaaaacatctattacttcgatgataactatcgtggtgcggtggaatggaaagaactggatggcgaaatgcattatttttctccggaaaccggtaaagcgtttaaaggcctgaaccagatcggcgattacaaatactacttcaacagcgatggcgtgatgcagaaaggctttgtgagcatcaacgataacaaacactatttcgatgatagcggtgtgatgaaagtgggctataccgaaattgatggcaaacatttctacttcgcggaaaacggcgaaatgcagattggcgtgttcaataccgaagatggtttcaaatacttcgcgcaccataacgaagatctgggtaacgaagaaggcgaagaaattagctatagcggcatcctgaacttcaacaacaaaatctactactttgatgatagctttaccgcggtggtgggctggaaagatctggaagatggcagcaaatattatttcgatgaagataccgcggaagcgtatattggcctgagcctgattaacgatggccagtactattttaacgatgatggcattatgcaggtgggtttcgtgaccattaatgataaagtgttctatttcagcgatagcggcattattgaaagcggcgtgcagaacattgatgataactacttctacatcgatgataacggcattgtgcagatcggcgtttttgataccagcgatggctacaaatatttcgcaccggccaataccgtgaacgataacatttatggccaggcggtggaatatagcggtctggtgcgtgtgggcgaagatgtgtattatttcggcgaaacctataccatcgaaaccggctggatttatgatatggaaaacgaaagcgataaatattactttaatccggaaacgaaaaaagcgtgcaaaggcattaacctgatcgatgatatcaaatactattttgatgaaaaaggcattatgcgtaccggtctgattagcttcgaaaacaacaactattacttcaacgaaaacggtgaaatgcagttcggctacatcaacatcgaagataaaatgttctacttcggcgaagatggtgttatgcagattggtgtttttaacaccccggatggcttcaaatactttgcccatcagaataccctggatgaaaatttcgaaggtgaaagcattaactataccggctggctggatctggatgaaaaacgctactacttcaccgatgaatacattgcggcgaccggcagcgtgattattgatggcgaagaatactacttcgatccggataccgcgcagctggtgattagcgaacatcatcatcatcaccat

SEQ ID NO: 25 - protein, 1129 aa, Clostridium Difficile
MATGWQTIDGKKYYFNTNTAIASTGYTIINGKHFYFNTDGIMQIGVFKGPNGFEYFAPANTDANNIEGQAILYQNEFLTLNGKKYYFGSDSKAVTGWRIINNKKYYFNPNNAIAAIHLCTINNDKYYFSYDGILQNGYITIERNNFYFDANNESKMVTGVFKGPNGFEYFAPANTHNNNIEGQAIVYQNKFLTLNGKKYYFDNDSKAVTGWQTIDGKKYYFNLNTAEAATGWQTIDGKKYYFNLNTAEAATGWQTIDGKKYYFNTNTFIASTGYTSINGKHFYFNTDGIMQIGVFKGPNGFEYFAPANTDANNIEGQAILYQNKFLTLNGKKYYFGSDSKAVTGLRTIDGKKYYFNTNTAVAVTGWQTINGKKYYFNTNTSIASTGYTIISGKHFYFNTDGIMQIGVFKGPDGFEYFAPANTDANNIEGQAIRYQNRFLYLHDNIYYFGNNSKAATGWVTIDGNRYYFEPNTAMGANGYKTIDNKNFYFRNGLPQIGVFKGSNGFEYFAPANTDANNIEGQAIRYQNRFLHLLGKIYYFGNNSKAVTGWQTINGKVYYFMPDTAMAAAGGLFEIDGVIYFFGVDGVKAVSGLIYINDSLYYFKPPVNNLITGFVTVGDDKYYFNPINGGAASIGETIIDDKNYYFNQSGVLQTGVFSTEDGFKYFAPANTLDENLEGEAIDFTGKLIIDENIYYFDDNYRGAVEWKELDGEMHYFSPETGKAFKGLNQIGDYKYYFNSDGVMQKGFVSINDNKHYFDDSGVMKVGYTEIDGKHFYFAENGEMQIGVFNTEDGFKYFAHHNEDLGNEEGEEISYSGILNFNNKIYYFDDSFTAVVGWKDLEDGSKYYFDEDTAEAYIGLSLINDGQYYFNDDGIMQVGFVTINDKVFYFSDSGIIESGVQNIDDNYFYIDDNGIVQIGVFDTSDGYKYFAPANTVNDNIYGQAVEYSGLVRVGEDVYYFGETYTIETGWIYDMENESDKYYFNPETKKACKGINLIDDIKYYFDEKGIMRTGLISFENNNYYFNENGEMQFGYINIEDKMFYFGEDGVMQIGVFNTPDGFKYFAHQNTLDENFEGESINYTGWLDLDEKRYYFTDEYIAATGSVIIDGEEYYFDPDTAQLVISEHHHHHH

SEQ ID NO: 26 - DNA, 2985 bp, Clostridium Difficile
atggcaaccggttggcagaccatcgatggcaaaaaatattattttaataccaacaccgcaattgcaagcaccggctataccattatcaacggcaaacacttttattttaacaccgacggcattatgcagattggtgtgtttaaaggtccgaacggctttgaatactttgcaccggcaaataccgatgccaataatattgaaggccaggccattctgtatcagaatgaatttctgaccctgaacggcaaaaaatactactttggcagcgatagcaaagcagttaccggttggcgcatcatcaacaataagaaatattacttcaacccgaataatgcaattgcagcaattcatctgtgcaccattaacaacgacaaatattatttcagctatgacggtattctgcagaatggctacattaccatcgaacgcaacaacttttatttcgatgccaacaacgaaagcaaaatggtgaccggtgttttcaaaggccctaatggttttgagtatttcgctccggcaaacacccataataacaacattgaaggtcaggcgatcgtttatcagaacaaattcctgacgctgaatggtaagaaatactatttcgataatgacagcaaagccgtgaccggctggcagacaattgacgggaagaaatattactttaatctgaataccgcagaagcagcaaccggttggcaaacgatcgacggtaaaaagtactacttcaacctgaacacagccgaagcagccacaggatggcagactattgatggaaaaaaatactatttcaacaccaacacctttattgcatctaccggttataccagcattaacggtaaacatttctacttcaacaccgatggtatcatgcagatcggcgttttcaaaggtccaaatggtttcgaatactttgcccctgccaatacagatgcaaataacatcgagggtcaggcaatcctgtaccaaaacaaatttctgaccctgaatgggaaaaaatattactttggtagcgattctaaagccgttaccggtctgcgtaccattgatggtaaaaaatactactttaatacgaatacagccgttgcggttacaggctggcagaccattaacgggaaaaaatactattttaacacaaataccagcattgcctcaacgggttataccattatttcgggtaaacacttctactttaataccgatggtattatgcaaatcggagtctttaaaggacctgatgggttcgaatattttgcgcctgcgaacactgatgcgaacaatatcgaaggacaggcaatccgctatcagaatcgctttctgtatctgcacgacaacatctattattttggcaacaattcaaaagcagccaccggctgggttacaattgatggcaaccgctactatttcgaaccgaataccgcaatgggtgcaaatggctacaaaaccatcgataataaaaatttctattttcgcaacggtctgccgcagatcggggtatttaaaggtagcaacggcttcgaatacttcgctccagcgaatacggacgcgaacaatattgagggtcaagcgattcgttatcaaaaccgttttctgcatctgctgggcaaaatctactactttggcaataacagtaaagcagttactggatggcagacaatcaatggtaaagtgtactattttatgccggataccgccatggcagcagccggtggtctgtttgaaattgatggcgtgatctatttttttggtgtggatggtgttaaagcagtgaaaggcctgaaccagatcggcgattacaaatactacttcaacagcgatggcgtgatgcagaaaggctttgtgagcatcaacgataacaaacactatttcgatgatagcggtgtgatgaaagtgggctataccgaaattgatggcaaacatttctacttcgcggaaaacggcgaaatgcagattggcgtgttcaataccgaagatggtttcaaatacttcgcgcaccataacgaagatctgggtaacgaagaaggcgaagaaattagctatagcggcatcctgaacttcaacaacaaaatctactactttgatgatagctttaccgcggtggtgggctggaaagatctggaagatggcagcaaatattatttcgatgaagataccgcggaagcgtatattggcctgagcctgattaacgatggccagtactattttaacgatgatggcattatgcaggtgggtttcgtgaccattaatgataaagtgttctatttcagcgatagcggcattattgaaagcggcgtgcagaacattgatgataactacttctacatcgatgataacggcattgtgcagatcggcgtttttgataccagcgatggctacaaatatttcgcaccggccaataccgtgaacgataacatttatggccaggcggtggaatatagcggtctggtgcgtgtgggcgaagatgtgtattatttcggcgaaacctataccatcgaaaccggctggatttatgatatggaaaacgaaagcgataaatattactttaatccggaaacgaaaaaagcgtgcaaaggcattaacctgatcgatgatatcaaatactattttgatgaaaaaggcattatgcgtaccggtctgattagcttcgaaaacaacaactattacttcaacgaaaacggtgaaatgcagttcggctacatcaacatcgaagataaaatgttctacttcggcgaagatggtgttatgcagattggtgtttttaacaccccggatggcttcaaatactttgcccatcagaataccctggatgaaaatttcgaaggtgaaagcattaactataccggctggctggatctggatgaaaaacgctactacttcaccgatgaatacattgcggcgaccggcagcgtgattattgatggcgaagaatactacttcgatccggataccgcgcagctggtgattagcgaacatcatcatcatcaccat

SEQ ID NO: 27 - protein, 995 aa, Clostridium Difficile
MATGWQTIDGKKYYFNTNTAIASTGYTIINGKHFYFNTDGIMQIGVFKGPNGFEYFAPANTDANNIEGQAILYQNEFLTLNGKKYYFGSDSKAVTGWRIINNKKYYFNPNNAIAAIHLCTINNDKYYFSYDGILQNGYITIERNNFYFDANNESKMVTGVFKGPNGFEYFAPANTHNNNIEGQAIVYQNKFLTLNGKKYYFDNDSKAVTGWQTIDGKKYYFNLNTAEAATGWQTIDGKKYYFNLNTAEAATGWQTIDGKKYYFNTNTFIASTGYTSINGKHFYFNTDGIMQIGVFKGPNGFEYFAPANTDANNIEGQAILYQNKFLTLNGKKYYFGSDSKAVTGLRTIDGKKYYFNTNTAVAVTGWQTINGKKYYFNTNTSIASTGYTIISGKHFYFNTDGIMQIGVFKGPDGFEYFAPANTDANNIEGQAIRYQNRFLYLHDNIYYFGNNSKAATGWVTIDGNRYYFEPNTAMGANGYKTIDNKNFYFRNGLPQIGVFKGSNGFEYFAPANTDANNIEGQAIRYQNRFLHLLGKIYYFGNNSKAVTGWQTINGKVYYFMPDTAMAAAGGLFEIDGVIYFFGVDGVKAVKGLNQIGDYKYYFNSDGVMQKGFVSINDNKHYFDDSGVMKVGYTEIDGKHFYFAENGEMQIGVFNTEDGFKYFAHHNEDLGNEEGEEISYSGILNFNNKIYYFDDSFTAVVGWKDLEDGSKYYFDEDTAEAYIGLSLINDGQYYFNDDGIMQVGFVTINDKVFYFSDSGIIESGVQNIDDNYFYIDDNGIVQIGVFDTSDGYKYFAPANTVNDNIYGQAVEYSGLVRVGEDVYYFGETYTIETGWIYDMENESDKYYFNPETKKACKGINLIDDIKYYFDEKGIMRTGLISFENNNYYFNENGEMQFGYINIEDKMFYFGEDGVMQIGVFNTPDGFKYFAHQNTLDENFEGESINYTGWLDLDEKRYYFTDEYIAATGSVIIDGEEYYFDPDTAQLVISEHHHHHH

SEQ ID NO: 28 - protein, 593 aa, Clostridium Difficile
MATGWQTIDGKKYYFNTNTAIASTGYTIINGKHFYFNTDGIMQIGVFKGPNGFEYFAPANTDANNIEGQAILYQNEFLTLNGKKYYFGSDSKAVTGWRIINNKKYYFNPNNAIAAIHLCTINNDKYYFSYDGILQNGYITIERNNFYFDANNESKMVTGVFKGPNGFEYFAPANTHNNNIEGQAIVYQNKFLTLNGKKYYFDNDSKAVTGWQTIDGKKYYFNLNTAEAATGWQTIDGKKYYFNLNTAEAATGWQTIDGKKYYFNTNTFIASTGYTSINGKHFYFNTDGIMQIGVFKGPNGFEYFAPANTDANNIEGQAILYQNKFLTLNGKKYYFGSDSKAVTGLRTIDGKKYYFNTNTAVAVTGWQTINGKKYYFNTNTSIASTGYTIISGKHFYFNTDGIMQIGVFKGPDGFEYFAPANTDANNIEGQAIRYQNRFLYLHDNIYYFGNNSKAATGWVTIDGNRYYFEPNTAMGANGYKTIDNKNFYFRNGLPQIGVFKGSNGFEYFAPANTDANNIEGQAIRYQNRFLHLLGKIYYFGNNSKAVTGWQTINGKVYYFMPDTAMAAAGGLFEIDGVIYFFGVDGVKAPGIYG

SEQ ID NO: 29 - protein, 589 aa, Clostridium Difficile
MATGWQTIDGKKYYFNTNTAIASTGYTIINGKHFYFNTDGIMQIGVFKGPNGFEYFAPANTDANNIEGQAILYQNEFLTLNGKKYYFGSDSKAVTGWRIINNKKYYFNPNNAIAAIHLCTINNDKYYFSYDGILQNGYITIERNNFYFDANNESKMVTGVFKGPNGFEYFAPANTHNNNIEGQAIVYQNKFLTLNGKKYYFDNDSKAVTGWQTIDGKKYYFNLNTAEAATGWQTIDGKKYYFNLNTAEAATGWQTIDGKKYYFNTNTFIASTGYTSINGKHFYFNTDGIMQIGVFKGPNGFEYFAPANTDANNIEGQAILYQNKFLTLNGKKYYFGSDSKAVTGLRTIDGKKYYFNTNTAVAVTGWQTINGKKYYFNTNTSIASTGYTIISGKHFYFNTDGIMQIGVFKGPDGFEYFAPANTDANNIEGQAIRYQNRFLYLHDNIYYFGNNSKAATGWVTIDGNRYYFEPNTAMGANGYKTIDNKNFYFRNGLPQIGVFKGSNGFEYFAPANTDANNIEGQAIRYQNRFLHLLGKIYYFGNNSKAVTGWQTINGKVYYFMPDTAMAAAGGLFEIDGVIYFFGVDGVKAV

SEQ ID NO: 30 - protein, 589 aa, Clostridium Difficile; identical to SEQ ID NO: 29

SEQ ID NO: 31 - protein, 589 aa, Clostridium Difficile; identical to SEQ ID NO: 29

SEQ ID NO: 32 - protein, 513 aa, Clostridium Difficile
TGFVTVGDDKYYFNPINGGAASIGETIIDDKNYYFNQSGVLQTGVFSTEDGFKYFAPANTLDENLEGEAIDFTGKLIIDENIYYFDDNYRGAVEWKELDGEMHYFSPETGKAFKGLNQIGDYKYYFNSDGVMQKGFVSINDNKHYFDDSGVMKVGYTEIDGKHFYFAENGEMQIGVFNTEDGFKYFAHHNEDLGNEEGEEISYSGILNFNNKIYYFDDSFTAVVGWKDLEDGSKYYFDEDTAEAYIGLSLINDGQYYFNDDGIMQVGFVTINDKVFYFSDSGIIESGVQNIDDNYFYIDDNGIVQIGVFDTSDGYKYFAPANTVNDNIYGQAVEYSGLVRVGEDVYYFGETYTIETGWIYDMENESDKYYFNPETKKACKGINLIDDIKYYFDEKGIMRTGLISFENNNYYFNENGEMQFGYINIEDKMFYFGEDGVMQIGVFNTPDGFKYFAHQNTLDENFEGESINYTGWLDLDEKRYYFTDEYIAATGSVIIDGEEYYFDPDTAQLVISE

SEQ ID NO: 33 - protein, 513 aa, Clostridium Difficile; identical to SEQ ID NO: 32

SEQ ID NO: 34 - protein, 534 aa, Clostridium Difficile
SGLIYINDSLYYFKPPVNNLITGFVTVGDDKYYFNPINGGAASIGETIIDDKNYYFNQSGVLQTGVFSTEDGFKYFAPANTLDENLEGEAIDFTGKLIIDENIYYFDDNYRGAVEWKELDGEMHYFSPETGKAFKGLNQIGDYKYYFNSDGVMQKGFVSINDNKHYFDDSGVMKVGYTEIDGKHFYFAENGEMQIGVFNTEDGFKYFAHHNEDLGNEEGEEISYSGILNFNNKIYYFDDSFTAVVGWKDLEDGSKYYFDEDTAEAYIGLSLINDGQYYFNDDGIMQVGFVTINDKVFYFSDSGIIESGVQNIDDNYFYIDDNGIVQIGVFDTSDGYKYFAPANTVNDNIYGQAVEYSGLVRVGEDVYYFGETYTIETGWIYDMENESDKYYFNPETKKACKGINLIDDIKYYFDEKGIMRTGLISFENNNYYFNENGEMQFGYINIEDKMFYFGEDGVMQIGVFNTPDGFKYFAHQNTLDENFEGESINYTGWLDLDEKRYYFTDEYIAATGSVIIDGEEYYFDPDTAQLVISE

SEQ ID NO: 35 - protein, 400 aa, Clostridium Difficile
KGLNQIGDYKYYFNSDGVMQKGFVSINDNKHYFDDSGVMKVGYTEIDGKHFYFAENGEMQIGVFNTEDGFKYFAHHNEDLGNEEGEEISYSGILNFNNKIYYFDDSFTAVVGWKDLEDGSKYYFDEDTAEAYIGLSLINDGQYYFNDDGIMQVGFVTINDKVFYFSDSGIIESGVQNIDDNYFYIDDNGIVQIGVFDTSDGYKYFAPANTVNDNIYGQAVEYSGLVRVGEDVYYFGETYTIETGWIYDMENESDKYYFNPETKKACKGINLIDDIKYYFDEKGIMRTGLISFENNNYYFNENGEMQFGYINIEDKMFYFGEDGVMQIGVFNTPDGFKYFAHQNTLDENFEGESINYTGWLDLDEKRYYFTDEYIAATGSVIIDGEEYYFDPDTAQLVISE